European Patent Specification EP 3 935 184 B1, published September 11, 2024. Title: COMPOSITIONS AND METHODS OF TARGETED NUCLEIC ACID ENRICHMENT BY LOOP ADAPTER PROTECTION AND EXONUCLEASE DIGESTION. Applicant: KING ABDULLAH UNIVERSITY OF SCIENCE AND TECHNOLOGY LI, MO BI, CHONGWEI WANG, LIN. The sequence listing filed with the application follows.

SEQUENCE LISTING (3 sequences)

SEQ ID NO: 1 - DNA, 26 bp, Artificial Sequence
  synthetic polynucleotide
  misc_feature (1)..(4): n is a, c, g, or t
nnnncagtccaggcttgcctggactg

SEQ ID NO: 2 - DNA, 9 bp, Artificial Sequence
  synthetic polynucleotide
cagtccagg

SEQ ID NO: 3 - DNA, 9 bp, Artificial Sequence
  synthetic polynucleotide
cctggactg